European Patent Application EP 4 807 365 A1, published September 16, 2026. Title: METHOD OF TREATING A SAMPLE. Applicant: MinervaX ApS. The sequence listing filed with the application follows.

SEQUENCE LISTING (32 sequences)

SEQ ID NO: 1 - protein, 332 aa, Lachnoanaerobaculum umeaense
NIVESDQDKANRIKSSLTTVKNDNVVQYTNEDGEIRTIIWAKGINGPTMGEGGDFHKEITNAGSDTYIDYKTSFTTGDGWYDVNKTRAGGNVDVDKNLCFGAVSSNMLHWWFEQNIEYIDRYIVKNGDIIRANRKISDLKYSFKSQQNSAIFELFKVLFGNNEKGFYTDLLMDLFINGYTPKTGGGTNIERDDLTPDSRGGFFYDVFKGEKLTDRTYGGSYEALGDKLKEVLGEAGLIGISHKAFKNSNHIVTLWGAEYDLNGKLIAVYISDSDDQNETEDERDLGMKRYEVRNVGGVAKLSTNQTNKSSGSAIGYLHILYLGTTQWENYFK

SEQ ID NO: 2 - protein, 682 aa, Lachnoanaerobaculum umeaense
MKKFNGKSVFLGLAAATIISSNAYAGIEGWKFEGNNWKYYKEDKALKAWQQLNNKWYFFNEDGSLKTGWHLDATNNWYFLDSSKNSNEGMLLSGWQWIDGYCYYFENIDKSTLGRMYVNTVVNGYRIDATGRWTNEKGVEYYEAGKGIITVNTLQGSLNTGKKSSGGGSSGKGGGLGKSGESGKGGSSIGGIGGKTGINQGDNNDTSNQSLIVEENSTVNNADQTKSVEKTKGDQKSEQNNSNEVNTTEGGQNKSGMTNNTSEYTYNKPTVNKENEDEKTNTTQDNKVSDSTSNDLSKTKDTQTNTNDSDIKSATASNAEIQKEEEHKNTETTNSSEKNKNTEQQNKSEENIVESDQDKANRIKSSLTTVKNDNVVQYTNEDGEIRTIIWAKGINGPTMGEGGDFHKEITNAGSDTYIDYKTSFTTGDGWYDVNKTRAGGNVDVDKNLCFGAVSSNMLHWWFEQNIEYIDRYIVKNGDIIRANRKISDLKYSFKSQQNSAIFELFKVLFGNNEKGFYTDLLMDLFINGYTPKTGGGTNIERDDLTPDSRGGFFYDVFKGEKLTDRTYGGSYEALGDKLKEVLGEAGLIGISHKAFKNSNHIVTLWGAEYDLNGKLIAVYISDSDDQNETEDERDLGMKRYEVRNVGGVAKLSTNQTNKSSGSAIGYLHILYLGTTQWENYFK

SEQ ID NO: 3 - protein, 664 aa, Lachnoanaerobaculum umeaense
MGIEGWKFEGNNWKYYKEDKALKAWQQLNNKWYFFNEDGSLKTGWHLDATNNWYFLDSSKNSNEGMLLSGWQWIDGYCYYFENIDKSTLGRMYVNTVVNGYRIDATGRWTNEKGVEYYEAGKGIITVNTLQGSLNTGKKSSGGGSSGKGGGLGKSGESGKGGSSIGGIGGKTGINQGDNNDTSNQSLIVEENSTVNNADQTKSVEKTKGDQKSEQNNSNEVNTTEGGQNKSGMTNNTSEYTYNKPTVNKENEDEKTNTTQDNKVSDSTSNDLSKTKDTQTNTNDSDIKSATASNAEIQKEEEHKNTETTNSSEKNKNTEQQNKSEENIVESDQDKANRIKSSLTTVKNDNVVQYTNEDGEIRTIIWAKGINGPTMGEGGDFHKEITNAGSDTYIDYKTSFTTGDGWYDVNKTRAGGNVDVDKNLCFGAVSSNMLHWWFEQNIEYIDRYIVKNGDIIRANRKISDLKYSFKSQQNSAIFELFKVLFGNNEKGFYTDLLMDLFINGYTPKTGGGTNIERDDLTPDSRGGFFYDVFKGEKLTDRTYGGSYEALGDKLKEVLGEAGLIGISHKAFKNSNHIVTLWGAEYDLNGKLIAVYISDSDDQNETEDERDLGMKRYEVRNVGGVAKLSTNQTNKSSGSAIGYLHILYLGTTQWENYFKHHHHHH

SEQ ID NO: 4 - protein, 668 aa, Lachnoanaerobaculum umeaense
MHHHHHHHHHHGIEGWKFEGNNWKYYKEDKALKAWQQLNNKWYFFNEDGSLKTGWHLDATNNWYFLDSSKNSNEGMLLSGWQWIDGYCYYFENIDKSTLGRMYVNTVVNGYRIDATGRWTNEKGVEYYEAGKGIITVNTLQGSLNTGKKSSGGGSSGKGGGLGKSGESGKGGSSIGGIGGKTGINQGDNNDTSNQSLIVEENSTVNNADQTKSVEKTKGDQKSEQNNSNEVNTTEGGQNKSGMTNNTSEYTYNKPTVNKENEDEKTNTTQDNKVSDSTSNDLSKTKDTQTNTNDSDIKSATASNAEIQKEEEHKNTETTNSSEKNKNTEQQNKSEENIVESDQDKANRIKSSLTTVKNDNVVQYTNEDGEIRTIIWAKGINGPTMGEGGDFHKEITNAGSDTYIDYKTSFTTGDGWYDVNKTRAGGNVDVDKNLCFGAVSSNMLHWWFEQNIEYIDRYIVKNGDIIRANRKISDLKYSFKSQQNSAIFELFKVLFGNNEKGFYTDLLMDLFINGYTPKTGGGTNIERDDLTPDSRGGFFYDVFKGEKLTDRTYGGSYEALGDKLKEVLGEAGLIGISHKAFKNSNHIVTLWGAEYDLNGKLIAVYISDSDDQNETEDERDLGMKRYEVRNVGGVAKLSTNQTNKSSGSAIGYLHILYLGTTQWENYFK

SEQ ID NO: 5 - protein, 438 aa, Lachnoanaerobaculum umeaense
MQNKSGMTNNTSEYTYNKPTVNKENEDEKTNTTQDNKVSDSTSNDLSKTKDTQTNTNDSDIKSATASNAEIQKEEEHKNTETTNSSEKNKNTEQQNKSEENIVESDQDKANRIKSSLTTVKNDNVVQYTNEDGEIRTIIWAKGINGPTMGEGGDFHKEITNAGSDTYIDYKTSFTTGDGWYDVNKTRAGGNVDVDKNLCFGAVSSNMLHWWFEQNIEYIDRYIVKNGDIIRANRKISDLKYSFKSQQNSAIFELFKVLFGNNEKGFYTDLLMDLFINGYTPKTGGGTNIERDDLTPDSRGGFFYDVFKGEKLTDRTYGGSYEALGDKLKEVLGEAGLIGISHKAFKNSNHIVTLWGAEYDLNGKLIAVYISDSDDQNETEDERDLGMKRYEVRNVGGVAKLSTNQTNKSSGSAIGYLHILYLGTTQWENYFKHHHHHH

SEQ ID NO: 6 - protein, 403 aa, Lachnoanaerobaculum umeaense
MSDSTSNDLSKTKDTQTNTNDSDIKSATASNAEIQKEEEHKNTETTNSSEKNKNTEQQNKSEENIVESDQDKANRIKSSLTTVKNDNVVQYTNEDGEIRTIIWAKGINGPTMGEGGDFHKEITNAGSDTYIDYKTSFTTGDGWYDVNKTRAGGNVDVDKNLCFGAVSSNMLHWWFEQNIEYIDRYIVKNGDIIRANRKISDLKYSFKSQQNSAIFELFKVLFGNNEKGFYTDLLMDLFINGYTPKTGGGTNIERDDLTPDSRGGFFYDVFKGEKLTDRTYGGSYEALGDKLKEVLGEAGLIGISHKAFKNSNHIVTLWGAEYDLNGKLIAVYISDSDDQNETEDERDLGMKRYEVRNVGGVAKLSTNQTNKSSGSAIGYLHILYLGTTQWENYFKLEHHHHHH

SEQ ID NO: 7 - protein, 339 aa, Lachnoanaerobaculum umeaense
MNIVESDQDKANRIKSSLTTVKNDNVVQYTNEDGEIRTIIWAKGINGPTMGEGGDFHKEITNAGSDTYIDYKTSFTTGDGWYDVNKTRAGGNVDVDKNLCFGAVSSNMLHWWFEQNIEYIDRYIVKNGDIIRANRKISDLKYSFKSQQNSAIFELFKVLFGNNEKGFYTDLLMDLFINGYTPKTGGGTNIERDDLTPDSRGGFFYDVFKGEKLTDRTYGGSYEALGDKLKEVLGEAGLIGISHKAFKNSNHIVTLWGAEYDLNGKLIAVYISDSDDQNETEDERDLGMKRYEVRNVGGVAKLSTNQTNKSSGSAIGYLHILYLGTTQWENYFKHHHHHH

SEQ ID NO: 8 - protein, 329 aa, Lachnoanaerobaculum gingivalis
AERKESTQNRAERFKESLITSENDNVVQYTNEDGEIRTIIWVKGINGPVMGEGGDFHKEITQGGKNTYVMYTVPYSSGDGWYDVNKTRSGGNIDIDKNLCFAAVSSNMLHWWFDQNIEYVDRYIEKNGDIIRANRKLSDLKTSFENPENSKIFELYKVLYGYNERGFYSDLLMDLFINGYTPNPKGGTNIESDDLIPNNNGGFFYDVFKGKKLTDRTYGGNYESLSNLLKEILGNGGIVGLSHKVFSKSNHIVTLWGAEYDLNGKLKAVYISDSDDQDESNVGMKRFEIRNVGGKAKISTNETDKSAGAELGYLHILYQGTGQWENYFK

SEQ ID NO: 9 - protein, 638 aa, Lachnoanaerobaculum gingivalis
MKKYKVGPVLLGLTMLMSFNAYAGVDGWKQENNSWKYYKEDKALKAWQQINNNWYFFNEDGSLKTGWYMDAANNWYFLDSSKTANEGVLLSGWQWIDGYCYYFEGIDNNTFGKMYSNTLVSGYKVDALGRWINESGAEYYEAGKGISTGNASQSSSNTAKKTSVAGSSEKSGKSGGSSKGGSSGKSGGSSKGGSSGKSGGSSFLNQGEKREENRILGESKGKAENSSSKRSEDLVGSRQDLSSDKNNSLIADNKTGNSEKAGSIEKNTNKEYTTKSNESPVKPATSSNVEIPKEEEKKDIESKESKKPEAERKESTQNRAERFKESLITSENDNVVQYTNEDGEIRTIIWVKGINGPVMGEGGDFHKEITQGGKNTYVMYTVPYSSGDGWYDVNKTRSGGNIDIDKNLCFAAVSSNMLHWWFDQNIEYVDRYIEKNGDIIRANRKLSDLKTSFENPENSKIFELYKVLYGYNERGFYSDLLMDLFINGYTPNPKGGTNIESDDLIPNNNGGFFYDVFKGKKLTDRTYGGNYESLSNLLKEILGNGGIVGLSHKVFSKSNHIVTLWGAEYDLNGKLKAVYISDSDDQDESNVGMKRFEIRNVGGKAKISTNETDKSAGAELGYLHILYQGTGQWENYFK

SEQ ID NO: 10 - protein, 622 aa, Lachnoanaerobaculum gingivalis
MGVDGWKQENNSWKYYKEDKALKAWQQINNNWYFFNEDGSLKTGWYMDAANNWYFLDSSKTANEGVLLSGWQWIDGYCYYFEGIDNNTFGKMYSNTLVSGYKVDALGRWINESGAEYYEAGKGISTGNASQSSSNTAKKTSVAGSSEKSGKSGGSSKGGSSGKSGGSSKGGSSGKSGGSSFLNQGEKREENRILGESKGKAENSSSKRSEDLVGSRQDLSSDKNNSLIADNKTGNSEKAGSIEKNTNKEYTTKSNESPVKPATSSNVEIPKEEEKKDIESKESKKPEAERKESTQNRAERFKESLITSENDNVVQYTNEDGEIRTIIWVKGINGPVMGEGGDFHKEITQGGKNTYVMYTVPYSSGDGWYDVNKTRSGGNIDIDKNLCFAAVSSNMLHWWFDQNIEYVDRYIEKNGDIIRANRKLSDLKTSFENPENSKIFELYKVLYGYNERGFYSDLLMDLFINGYTPNPKGGTNIESDDLIPNNNGGFFYDVFKGKKLTDRTYGGNYESLSNLLKEILGNGGIVGLSHKVFSKSNHIVTLWGAEYDLNGKLKAVYISDSDDQDESNVGMKRFEIRNVGGKAKISTNETDKSAGAELGYLHILYQGTGQWENYFKHHHHHH

SEQ ID NO: 11 - protein, 626 aa, Lachnoanaerobaculum gingivalis
MHHHHHHHHHHGVDGWKQENNSWKYYKEDKALKAWQQINNNWYFFNEDGSLKTGWYMDAANNWYFLDSSKTANEGVLLSGWQWIDGYCYYFEGIDNNTFGKMYSNTLVSGYKVDALGRWINESGAEYYEAGKGISTGNASQSSSNTAKKTSVAGSSEKSGKSGGSSKGGSSGKSGGSSKGGSSGKSGGSSFLNQGEKREENRILGESKGKAENSSSKRSEDLVGSRQDLSSDKNNSLIADNKTGNSEKAGSIEKNTNKEYTTKSNESPVKPATSSNVEIPKEEEKKDIESKESKKPEAERKESTQNRAERFKESLITSENDNVVQYTNEDGEIRTIIWVKGINGPVMGEGGDFHKEITQGGKNTYVMYTVPYSSGDGWYDVNKTRSGGNIDIDKNLCFAAVSSNMLHWWFDQNIEYVDRYIEKNGDIIRANRKLSDLKTSFENPENSKIFELYKVLYGYNERGFYSDLLMDLFINGYTPNPKGGTNIESDDLIPNNNGGFFYDVFKGKKLTDRTYGGNYESLSNLLKEILGNGGIVGLSHKVFSKSNHIVTLWGAEYDLNGKLKAVYISDSDDQDESNVGMKRFEIRNVGGKAKISTNETDKSAGAELGYLHILYQGTGQWENYFK

SEQ ID NO: 12 - DNA, 999 bp, Lachnoanaerobaculum umeaense
  source 1..999: mol_type = other DNA
aatatagtagagagtgatcaggataaggccaatagaataaaatcctctttgactaccgttaaaaatgataatgtggtacagtacacgaatgaagatggagaaattagaacaattatttgggcaaagggcatcaatggacctactatgggagagggtggagattttcacaaagaaataacaaatgcgggttcagatacatatatagattataaaacttcgttcactacaggtgatggatggtatgatgtaaataagacaagagccggtggcaatgtagacgtagataaaaatctttgctttggggcagtttcatccaatatgctacattggtggtttgaacaaaatattgaatatattgacagatatatagtaaagaatggagatataattcgtgcaaataggaagatctcagatctgaaatattcttttaagagtcagcaaaatagtgctatattcgaactctttaaggtgttatttggaaataatgagaagggattttatacagaccttttgatggacctgtttataaacggatatactccaaagacaggtggaggtacaaatatagaaagagatgatttaacacctgatagcagaggtggatttttctatgatgtgtttaaaggagagaagctgacagaccgtacttatggtggaagttatgaagctttaggtgataaattaaaagaagtactgggagaagccggtttgataggtatatctcataaggcttttaaaaacagtaatcatatagtaactctatggggtgctgaatatgatttgaatggaaagcttatagcggtatatattagtgattcagatgatcaaaatgaaacagaagatgaaagagatctgggcatgaaacgctatgaggttaggaatgtaggaggagtggcaaaactgtccacaaatcaaacgaataagtcgtcaggttcagctataggatatcttcatatactatacttaggaaccacacagtgggaaaattattttaaataa

SEQ ID NO: 13 - DNA, 2049 bp, Lachnoanaerobaculum umeaense
  source 1..2049: mol_type = other DNA
atgaaaaagtttaacggtaagtctgtttttttaggacttgcagcagcaactataatctcatctaatgcctatgcaggtattgaaggatggaaatttgagggtaataattggaaatattataaagaagataaagctttaaaggcctggcagcaattaaataataaatggtatttttttaatgaggatggaagtttaaaaacaggatggcatttggatgctacaaataattggtactttttagacagctctaaaaattctaatgaaggtatgcttttgtcaggatggcagtggatagacggatactgctattattttgaaaacattgataaatctactcttggcagaatgtatgtaaatactgtagtgaatggatatagaattgatgctacaggtagatggacaaatgaaaaaggtgttgaatattatgaagcaggcaagggaataattacagttaatactttacaaggctctttaaatacaggtaaaaaatcaagtggaggtggaagctccggtaaaggtggtggtttgggaaaaagcggagaatccggtaaaggtggatcaagtatagggggtattggtggaaaaaccggcataaatcaaggcgataataatgatacttcaaatcaaagcctgatagtagaagaaaattcgactgtgaataatgcagatcagactaagagtgtagaaaaaacaaagggtgatcaaaaatctgaacaaaataattcaaatgaagtaaatactactgaaggtggtcagaacaaatccggaatgactaataatacaagtgagtatacttataataaacctactgtgaataaagaaaatgaagatgaaaaaactaatacaacacaggataacaaagtatcggatagcacttcaaatgatttgagtaaaacaaaagatacacagacaaatacaaatgatagtgatataaagtcggctactgcttcaaatgccgaaatccaaaaggaagaagaacataaaaatacagaaactacgaatagttctgagaagaataaaaatactgaacagcagaacaaatctgaagagaatatagtagagagtgatcaggataaggccaatagaataaaatcctctttgactaccgttaaaaatgataatgtggtacagtacacgaatgaagatggagaaattagaacaattatttgggcaaagggcatcaatggacctactatgggagagggtggagattttcacaaagaaataacaaatgcgggttcagatacatatatagattataaaacttcgttcactacaggtgatggatggtatgatgtaaataagacaagagccggtggcaatgtagacgtagataaaaatctttgctttggggcagtttcatccaatatgctacattggtggtttgaacaaaatattgaatatattgacagatatatagtaaagaatggagatataattcgtgcaaataggaagatctcagatctgaaatattcttttaagagtcagcaaaatagtgctatattcgaactctttaaggtgttatttggaaataatgagaagggattttatacagaccttttgatggacctgtttataaacggatatactccaaagacaggtggaggtacaaatatagaaagagatgatttaacacctgatagcagaggtggatttttctatgatgtgtttaaaggagagaagctgacagaccgtacttatggtggaagttatgaagctttaggtgataaattaaaagaagtactgggagaagccggtttgataggtatatctcataaggcttttaaaaacagtaatcatatagtaactctatggggtgctgaatatgatttgaatggaaagcttatagcggtatatattagtgattcagatgatcaaaatgaaacagaagatgaaagagatctgggcatgaaacgctatgaggttaggaatgtaggaggagtggcaaaactgtccacaaatcaaacgaataagtcgtcaggttcagctataggatatcttcatatactatacttaggaaccacacagtgggaaaattattttaaataa

SEQ ID NO: 14 - DNA, 2001 bp, Lachnoanaerobaculum umeaense
  source 1..2001: mol_type = other DNA
atgggcatcgaaggttggaaattcgagggtaacaactggaagtactataaagaggataaggcgctgaaagcgtggcagcaactgaacaacaaatggtacttctttaacgaagacggcagcctgaagaccggttggcacctggatgcgaccaacaactggtatttcctggacagcagcaaaaacagcaacgagggcatgctgctgagcggttggcaatggatcgatggttactgctactacttcgaaaacatcgacaagagcaccctgggccgtatgtacgttaacaccgtggttaacggctatcgtatcgacgcgaccggtcgttggaccaacgagaaaggcgttgaatactatgaggcgggcaagggtatcattaccgtgaacaccctgcagggcagcctgaacaccggtaagaaaagcagcggtggcggtagcagcggcaagggcggtggcctgggcaaaagcggtgaaagcggcaagggtggcagcagcatcggtggcattggtggcaaaaccggcatcaaccagggtgacaacaacgataccagcaaccaaagcctgattgttgaggaaaacagcaccgtgaacaacgcggatcaaaccaaaagcgttgagaagaccaaaggtgaccagaagagcgaacaaaacaacagcaacgaagtgaacaccaccgagggtggccagaacaagagcggcatgaccaacaacaccagcgagtacacctataacaagccgaccgttaacaaagaaaacgaggatgaaaaaaccaacaccacccaggacaacaaagtgagcgatagcaccagcaacgacctgagcaagaccaaagacacccaaaccaacaccaacgacagcgatatcaaaagcgcgaccgcgagcaacgcggagattcagaaggaagaggagcacaaaaacaccgaaaccaccaacagcagcgagaagaacaaaaacaccgaacagcaaaacaagagcgaagagaacatcgttgaaagcgaccaagataaggcgaaccgtattaaaagcagcctgaccaccgtgaaaaacgataacgtggttcagtacaccaacgaagacggcgagatccgtaccatcatttgggcgaagggtattaacggcccgaccatgggcgagggtggcgatttccacaaagaaatcaccaacgcgggcagcgacacctacattgattataagaccagctttaccaccggcgacggttggtatgatgttaacaaaacccgtgcgggtggcaacgtggacgttgataagaacctgtgcttcggtgctgtgagcagcaacatgctgcactggtggtttgaacagaacatcgagtacattgatcgttatatcgttaaaaacggcgacatcattcgtgcgaaccgtaagattagcgacctgaagtacagcttcaaaagccagcaaaacagcgcgatcttcgagctgtttaaagtgctgttcggcaacaacgaaaagggtttttacaccgacctgctgatggacctgttcatcaacggttataccccgaaaaccggtggcggtaccaacattgagcgtgacgatctgaccccggatagccgtggcggtttcttttacgacgttttcaagggcgagaaactgaccgatcgtacctacggcggtagctatgaagcgctgggcgacaagctgaaagaagtgctgggcgaggcgggcctgatcggtattagccacaaggcgtttaaaaatagcaaccacatcgttaccctgtggggtgcggagtacgatctgaacggcaaactgatcgcggtgtatattagcgacagcgacgatcagaacgagaccgaagacgagcgtgatctgggtatgaagcgttacgaagtgcgtaacgttggcggtgtggcgaaactgagcaccaaccaaaccaacaagagcagcggcagcgcgatcggttacctgcacattctgtatctgggtaccacccagtgggaaaactatttcaagctcgagcaccaccaccaccaccactga

SEQ ID NO: 15 - DNA, 2013 bp, Lachnoanaerobaculum umeaense
  source 1..2013: mol_type = other DNA
atgcaccaccaccaccaccaccaccaccaccacggcatcgaaggttggaaattcgagggtaacaactggaagtactataaagaggataaggcgctgaaagcgtggcagcaactgaacaacaaatggtacttctttaacgaagacggcagcctgaagaccggttggcacctggatgcgaccaacaactggtatttcctggacagcagcaaaaacagcaacgagggcatgctgctgagcggttggcaatggatcgatggttactgctactacttcgaaaacatcgacaagagcaccctgggccgtatgtacgttaacaccgtggttaacggctatcgtatcgacgcgaccggtcgttggaccaacgagaaaggcgttgaatactatgaggcgggcaagggtatcattaccgtgaacaccctgcagggcagcctgaacaccggtaagaaaagcagcggtggcggtagcagcggcaagggcggtggcctgggcaaaagcggtgaaagcggcaagggtggcagcagcatcggtggcattggtggcaaaaccggcatcaaccagggtgacaacaacgataccagcaaccaaagcctgattgttgaggaaaacagcaccgtgaacaacgcggatcaaaccaaaagcgttgagaagaccaaaggtgaccagaagagcgaacaaaacaacagcaacgaagtgaacaccaccgagggtggccagaacaagagcggcatgaccaacaacaccagcgagtacacctataacaagccgaccgttaacaaagaaaacgaggatgaaaaaaccaacaccacccaggacaacaaagtgagcgatagcaccagcaacgacctgagcaagaccaaagacacccaaaccaacaccaacgacagcgatatcaaaagcgcgaccgcgagcaacgcggagattcagaaggaagaggagcacaaaaacaccgaaaccaccaacagcagcgagaagaacaaaaacaccgaacagcaaaacaagagcgaagagaacatcgttgaaagcgaccaagataaggcgaaccgtattaaaagcagcctgaccaccgtgaaaaacgataacgtggttcagtacaccaacgaagacggcgagatccgtaccatcatttgggcgaagggtattaacggcccgaccatgggcgagggtggcgatttccacaaagaaatcaccaacgcgggcagcgacacctacattgattataagaccagctttaccaccggcgacggttggtatgatgttaacaaaacccgtgcgggtggcaacgtggacgttgataagaacctgtgcttcggtgctgtgagcagcaacatgctgcactggtggtttgaacagaacatcgagtacattgatcgttatatcgttaaaaacggcgacatcattcgtgcgaaccgtaagattagcgacctgaagtacagcttcaaaagccagcaaaacagcgcgatcttcgagctgtttaaagtgctgttcggcaacaacgaaaagggtttttacaccgacctgctgatggacctgttcatcaacggttataccccgaaaaccggtggcggtaccaacattgagcgtgacgatctgaccccggatagccgtggcggtttcttttacgacgttttcaagggcgagaaactgaccgatcgtacctacggcggtagctatgaagcgctgggcgacaagctgaaagaagtgctgggcgaggcgggcctgatcggtattagccacaaggcgtttaaaaatagcaaccacatcgttaccctgtggggtgcggagtacgatctgaacggcaaactgatcgcggtgtatattagcgacagcgacgatcagaacgagaccgaagacgagcgtgatctgggtatgaagcgttacgaagtgcgtaacgttggcggtgtggcgaaactgagcaccaaccaaaccaacaagagcagcggcagcgcgatcggttacctgcacattctgtatctgggtaccacccagtgggaaaactatttcaagctcgagtga

SEQ ID NO: 16 - DNA, 1323 bp, Lachnoanaerobaculum umeaense
  source 1..1323: mol_type = other DNA
atgcagaacaagagcggcatgaccaacaacaccagcgagtacacctataacaagccgaccgttaacaaagaaaacgaggatgaaaaaaccaacaccacccaggacaacaaagtgagcgatagcaccagcaacgacctgagcaagaccaaagacacccaaaccaacaccaacgacagcgatatcaaaagcgcgaccgcgagcaacgcggagattcagaaggaagaggagcacaaaaacaccgaaaccaccaacagcagcgagaagaacaaaaacaccgaacagcaaaacaagagcgaagagaacatcgttgaaagcgaccaagataaggcgaaccgtattaaaagcagcctgaccaccgtgaaaaacgataacgtggttcagtacaccaacgaagacggcgagatccgtaccatcatttgggcgaagggtattaacggcccgaccatgggcgagggtggcgatttccacaaagaaatcaccaacgcgggcagcgacacctacattgattataagaccagctttaccaccggcgacggttggtatgatgttaacaaaacccgtgcgggtggcaacgtggacgttgataagaacctgtgcttcggtgctgtgagcagcaacatgctgcactggtggtttgaacagaacatcgagtacattgatcgttatatcgttaaaaacggcgacatcattcgtgcgaaccgtaagattagcgacctgaagtacagcttcaaaagccagcaaaacagcgcgatcttcgagctgtttaaagtgctgttcggcaacaacgaaaagggtttttacaccgacctgctgatggacctgttcatcaacggttataccccgaaaaccggtggcggtaccaacattgagcgtgacgatctgaccccggatagccgtggcggtttcttttacgacgttttcaagggcgagaaactgaccgatcgtacctacggcggtagctatgaagcgctgggcgacaagctgaaagaagtgctgggcgaggcgggcctgatcggtattagccacaaggcgtttaaaaatagcaaccacatcgttaccctgtggggtgcggagtacgatctgaacggcaaactgatcgcggtgtatattagcgacagcgacgatcagaacgagaccgaagacgagcgtgatctgggtatgaagcgttacgaagtgcgtaacgttggcggtgtggcgaaactgagcaccaaccaaaccaacaagagcagcggcagcgcgatcggttacctgcacattctgtatctgggtaccacccagtgggaaaactatttcaagctcgagcaccaccaccaccaccactga

SEQ ID NO: 17 - DNA, 1212 bp, Lachnoanaerobaculum umeaense
  source 1..1212: mol_type = other DNA
atgagcgatagcaccagcaacgacctgagcaagaccaaagacacccaaaccaacaccaacgacagcgatatcaaaagcgcgaccgcgagcaacgcggagattcagaaggaagaggagcacaaaaacaccgaaaccaccaacagcagcgagaagaacaaaaacaccgaacagcaaaacaagagcgaagagaacatcgttgaaagcgaccaagataaggcgaaccgtattaaaagcagcctgaccaccgtgaaaaacgataacgtggttcagtacaccaacgaagacggcgagatccgtaccatcatttgggcgaagggtattaacggcccgaccatgggcgagggtggcgatttccacaaagaaatcaccaacgcgggcagcgacacctacattgattataagaccagctttaccaccggcgacggttggtatgatgttaacaaaacccgtgcgggtggcaacgtggacgttgataagaacctgtgcttcggtgctgtgagcagcaacatgctgcactggtggtttgaacagaacatcgagtacattgatcgttatatcgttaaaaacggcgacatcattcgtgcgaaccgtaagattagcgacctgaagtacagcttcaaaagccagcaaaacagcgcgatcttcgagctgtttaaagtgctgttcggcaacaacgaaaagggtttttacaccgacctgctgatggacctgttcatcaacggttataccccgaaaaccggtggcggtaccaacattgagcgtgacgatctgaccccggatagccgtggcggtttcttttacgacgttttcaagggcgagaaactgaccgatcgtacctacggcggtagctatgaagcgctgggcgacaagctgaaagaagtgctgggcgaggcgggcctgatcggtattagccacaaggcgtttaaaaatagcaaccacatcgttaccctgtggggtgcggagtacgatctgaacggcaaactgatcgcggtgtatattagcgacagcgacgatcagaacgagaccgaagacgagcgtgatctgggtatgaagcgttacgaagtgcgtaacgttggcggtgtggcgaaactgagcaccaaccaaaccaacaagagcagcggcagcgcgatcggttacctgcacattctgtatctgggtaccacccagtgggaaaactatttcaagctcgagcaccaccaccaccaccactga

SEQ ID NO: 18 - DNA, 1026 bp, Lachnoanaerobaculum umeaense
  source 1..1026: mol_type = other DNA
atgaacatcgttgaaagcgaccaagataaggcgaaccgtattaaaagcagcctgaccaccgtgaaaaacgataacgtggttcagtacaccaacgaagacggcgagatccgtaccatcatttgggcgaagggtattaacggcccgaccatgggcgagggtggcgatttccacaaagaaatcaccaacgcgggcagcgacacctacattgattataagaccagctttaccaccggcgacggttggtatgatgttaacaaaacccgtgcgggtggcaacgtggacgttgataagaacctgtgcttcggtgctgtgagcagcaacatgctgcactggtggtttgaacagaacatcgagtacattgatcgttatatcgttaaaaacggcgacatcattcgtgcgaaccgtaagattagcgacctgaagtacagcttcaaaagccagcaaaacagcgcgatcttcgagctgtttaaagtgctgttcggcaacaacgaaaagggtttttacaccgacctgctgatggacctgttcatcaacggttataccccgaaaaccggtggcggtaccaacattgagcgtgacgatctgaccccggatagccgtggcggtttcttttacgacgttttcaagggcgagaaactgaccgatcgtacctacggcggtagctatgaagcgctgggcgacaagctgaaagaagtgctgggcgaggcgggcctgatcggtattagccacaaggcgtttaaaaatagcaaccacatcgttaccctgtggggtgcggagtacgatctgaacggcaaactgatcgcggtgtatattagcgacagcgacgatcagaacgagaccgaagacgagcgtgatctgggtatgaagcgttacgaagtgcgtaacgttggcggtgtggcgaaactgagcaccaaccaaaccaacaagagcagcggcagcgcgatcggttacctgcacattctgtatctgggtaccacccagtgggaaaactatttcaagctcgagcaccaccaccaccaccactga

SEQ ID NO: 19 - DNA, 990 bp, Lachnoanaerobaculum gingivalis
  source 1..990: mol_type = other DNA
gcagaaagaaaagagagtacacaaaacagggctgagagatttaaagaatcattaattacttcagagaatgacaatgttgttcagtatacaaatgaagacggtgaaatacgaaccatcatatgggtaaagggaattaacggacctgttatgggagaaggtggagactttcataaagagattacacaaggcggtaagaatacttatgtaatgtatactgtaccatattcaagcggagacggatggtatgatgttaataaaacaagaagcggtggaaatatcgatatagataaaaatctttgctttgcagcggtatcatcaaatatgcttcattggtggtttgatcaaaatattgaatatgttgacagatatatagaaaaaaacggagatataattcgtgccaacagaaaactttcagatttaaaaacttcctttgaaaatccggaaaacagtaaaatatttgagctgtataaagtattgtacggatataatgagagagggttttattcggatcttttgatggatttatttattaacggatatactccaaacccaaagggtggaacaaatatagaaagtgatgatcttatcccaaataataacggcggattcttctatgatgttttcaaggggaaaaaacttacagaccgtacttatggtggaaactatgaatcactaagtaatcttcttaaagaaatcttgggtaatggcggcatagtaggactttctcataaagtgttttcaaagagtaatcatatagttactttgtggggtgccgaatatgacttgaacgggaagttgaaggctgtatatataagcgattctgacgatcaggatgaaagtaatgtaggcatgaaacgttttgaaatccgaaatgtaggaggaaaagcaaaaatatctaccaacgaaacagataagtctgcgggtgctgaattaggatatcttcatatcctatatcagggaaccggacaatgggaaaattattttaaataa

SEQ ID NO: 20 - DNA, 1917 bp, Lachnoanaerobaculum gingivalis
  source 1..1917: mol_type = other DNA
atgaaaaaatataaagtcggtcctgtattgttgggacttactatgttgatgtcctttaatgcctatgcaggtgttgatggatggaaacaggaaaataacagttggaaatattataaagaagataaggctctaaaggcttggcagcagataaataataattggtatttctttaatgaagacggaagtttaaaaaccggttggtatatggacgccgcaaataattggtattttttagacagctctaaaactgccaatgagggagtgcttttatcaggatggcagtggatagacggatattgctattattttgagggaatagataataatacattcggaaagatgtattcaaatactcttgtcagcggatataaagttgatgctttaggaagatggattaatgaaagcggagcagaatattatgaagccggtaaaggtataagtacaggtaatgcttcacaaagttcatcgaatacagcaaagaaaacaagtgttgcaggaagttcggaaaaaagcggtaaaagcggaggctcaagcaagggcggaagctccggaaaaagcggaggctcaagcaagggcggaagttccggtaaaagcggaggctcaagctttttaaatcaaggagaaaaaagagaagaaaacagaatattaggagaatcaaaaggaaaggctgaaaactcaagttccaaaagaagtgaagacttggtaggttcaagacaagacttaagctcggataaaaataacagcttgattgcagataataaaacaggaaatagtgagaaagccggaagcatagaaaaaaatacaaataaagagtataccacaaagtcaaatgagagccctgtaaaaccggccacttcctcaaatgtcgagataccgaaagaagaggaaaaaaaggatatagagtcaaaggaaagtaaaaagcctgaggcagaaagaaaagagagtacacaaaacagggctgagagatttaaagaatcattaattacttcagagaatgacaatgttgttcagtatacaaatgaagacggtgaaatacgaaccatcatatgggtaaagggaattaacggacctgttatgggagaaggtggagactttcataaagagattacacaaggcggtaagaatacttatgtaatgtatactgtaccatattcaagcggagacggatggtatgatgttaataaaacaagaagcggtggaaatatcgatatagataaaaatctttgctttgcagcggtatcatcaaatatgcttcattggtggtttgatcaaaatattgaatatgttgacagatatatagaaaaaaacggagatataattcgtgccaacagaaaactttcagatttaaaaacttcctttgaaaatccggaaaacagtaaaatatttgagctgtataaagtattgtacggatataatgagagagggttttattcggatcttttgatggatttatttattaacggatatactccaaacccaaagggtggaacaaatatagaaagtgatgatcttatcccaaataataacggcggattcttctatgatgttttcaaggggaaaaaacttacagaccgtacttatggtggaaactatgaatcactaagtaatcttcttaaagaaatcttgggtaatggcggcatagtaggactttctcataaagtgttttcaaagagtaatcatatagttactttgtggggtgccgaatatgacttgaacgggaagttgaaggctgtatatataagcgattctgacgatcaggatgaaagtaatgtaggcatgaaacgttttgaaatccgaaatgtaggaggaaaagcaaaaatatctaccaacgaaacagataagtctgcgggtgctgaattaggatatcttcatatcctatatcagggaaccggacaatgggaaaattattttaaataa

SEQ ID NO: 21 - DNA, 1875 bp, Lachnoanaerobaculum gingivalis
  source 1..1875: mol_type = other DNA
atgggtgtggacggctggaaacaggagaacaacagctggaagtactataaagaagataaggcgctgaaagcgtggcagcaaatcaacaacaactggtatttctttaacgaggacggtagcctgaaaaccggctggtacatggacgcggcgaacaactggtatttcctggatagcagcaagaccgcgaacgagggtgttctgctgagcggctggcagtggatcgacggttactgctactatttcgaaggcattgataacaacacctttggtaaaatgtacagcaacaccctggttagcggctataaggttgacgcgctgggtcgttggatcaacgagagcggcgcggaatactatgaggcgggtaaaggcattagcaccggtaacgcgagccaaagcagcagcaacaccgcgaagaaaaccagcgtggcgggtagcagcgaaaagagcggcaaaagcggtggcagcagcaagggtggcagcagcggtaagagcggtggcagcagcaagggtggcagcagcgggaaaagcggtggcagcagcttcctgaaccagggcgagaagcgtgaggaaaaccgtatcctgggtgaaagcaagggcaaagcggagaacagcagcagcaaacgtagcgaagacctggttggtagccgtcaagacctgagcagcgataagaacaacagcctgatcgcggataacaagaccggtaacagcgaaaaagcgggcagcattgagaagaacaccaacaaagaatataccaccaagagcaacgagagcccggtgaaaccggcgaccagcagcaacgttgaaatcccgaaggaagaggagaagaaggacattgaaagcaaagagagcaagaaaccggaagcggagcgtaaggagagcacccagaaccgtgcggaacgtttcaaagagagcctgatcaccagcgaaaacgacaacgtggttcaatataccaacgaagatggcgagatccgtaccatcatttgggtgaagggtattaacggcccggttatgggcgagggtggcgattttcacaaggaaattacccagggtggcaaaaacacctacgtgatgtataccgttccgtacagcagcggtgacggctggtatgatgtgaacaaaacccgtagcggtggcaacatcgacattgataagaacctgtgcttcgcggctgtgagcagcaacatgctgcactggtggtttgaccaaaacatcgagtacgttgatcgttatattgagaagaacggtgacatcattcgtgcgaaccgtaagctgagcgatctgaaaaccagcttcgaaaacccggagaacagcaagatctttgagctgtacaaagtgctgtacggttataacgaacgtggcttctatagcgacctgctgatggacctgttcattaacggttacaccccgaacccgaagggtggcaccaacatcgagagcgacgatctgattccgaacaacaacggtggcttcttttacgacgttttcaaaggcaagaaactgaccgatcgtacctacggtggcaactatgagagcctgagcaacctgctgaaggaaatcctgggtaacggtggcattgtgggcctgagccacaaggtttttagcaaaagcaaccacatcgtgaccctgtggggtgcggagtacgacctgaacggcaagctgaaagcggtttatattagcgacagcgacgatcaagatgagagcaacgtgggtatgaaacgtttcgaaatccgtaacgttggtggcaaggcgaaaattagcaccaacgagaccgataagagcgcgggtgcggaactgggctacctgcacatcctgtatcagggtaccggccaatgggaaaactactttaagctcgagcaccaccaccaccaccactga

SEQ ID NO: 22 - DNA, 1887 bp, Lachnoanaerobaculum gingivalis
  source 1..1887: mol_type = other DNA
atgcaccaccaccaccaccaccaccaccaccacggtgtggacggctggaaacaggagaacaacagctggaagtactataaagaagataaggcgctgaaagcgtggcagcaaatcaacaacaactggtatttctttaacgaggacggtagcctgaaaaccggctggtacatggacgcggcgaacaactggtatttcctggatagcagcaagaccgcgaacgagggtgttctgctgagcggctggcagtggatcgacggttactgctactatttcgaaggcattgataacaacacctttggtaaaatgtacagcaacaccctggttagcggctataaggttgacgcgctgggtcgttggatcaacgagagcggcgcggaatactatgaggcgggtaaaggcattagcaccggtaacgcgagccaaagcagcagcaacaccgcgaagaaaaccagcgtggcgggtagcagcgaaaagagcggcaaaagcggtggcagcagcaagggtggcagcagcggtaagagcggtggcagcagcaagggtggcagcagcgggaaaagcggtggcagcagcttcctgaaccagggcgagaagcgtgaggaaaaccgtatcctgggtgaaagcaagggcaaagcggagaacagcagcagcaaacgtagcgaagacctggttggtagccgtcaagacctgagcagcgataagaacaacagcctgatcgcggataacaagaccggtaacagcgaaaaagcgggcagcattgagaagaacaccaacaaagaatataccaccaagagcaacgagagcccggtgaaaccggcgaccagcagcaacgttgaaatcccgaaggaagaggagaagaaggacattgaaagcaaagagagcaagaaaccggaagcggagcgtaaggagagcacccagaaccgtgcggaacgtttcaaagagagcctgatcaccagcgaaaacgacaacgtggttcaatataccaacgaagatggcgagatccgtaccatcatttgggtgaagggtattaacggcccggttatgggcgagggtggcgattttcacaaggaaattacccagggtggcaaaaacacctacgtgatgtataccgttccgtacagcagcggtgacggctggtatgatgtgaacaaaacccgtagcggtggcaacatcgacattgataagaacctgtgcttcgcggctgtgagcagcaacatgctgcactggtggtttgaccaaaacatcgagtacgttgatcgttatattgagaagaacggtgacatcattcgtgcgaaccgtaagctgagcgatctgaaaaccagcttcgaaaacccggagaacagcaagatctttgagctgtacaaagtgctgtacggttataacgaacgtggcttctatagcgacctgctgatggacctgttcattaacggttacaccccgaacccgaagggtggcaccaacatcgagagcgacgatctgattccgaacaacaacggtggcttcttttacgacgttttcaaaggcaagaaactgaccgatcgtacctacggtggcaactatgagagcctgagcaacctgctgaaggaaatcctgggtaacggtggcattgtgggcctgagccacaaggtttttagcaaaagcaaccacatcgtgaccctgtggggtgcggagtacgacctgaacggcaagctgaaagcggtttatattagcgacagcgacgatcaagatgagagcaacgtgggtatgaaacgtttcgaaatccgtaacgttggtggcaaggcgaaaattagcaccaacgagaccgataagagcgcgggtgcggaactgggctacctgcacatcctgtatcagggtaccggccaatgggaaaactactttaagctcgagtga

SEQ ID NO: 23 - protein, 629 aa, Lachnoanaerobaculum sp. ICM7
MLMSFNAYAGADGWKQENNKWKYYKEDKALKAWQQINNNWYFFNEDGSLKTGWYMDASNNWYFLDSSKTANEGVLLSGWQWIDGYCYYFEGTDNTTFGKMYSNTDVSGYRVDALGRWINESGTEYYEAGKGISTGNASQSSSNTAKKQGNAGGLGKSSGSGGLGKGESSGKGGSSGKSRGLGRGGSLGKDGGSDSLGKGESYDKSAGSNKGENTGRSDDLSNLNQGEKREESRILRESENGGSFSRSEGSISQRKELSQDKEDTQKSNESPVKPATSSNVEIPKEEEKKDIEPKESKKLEAKRKESTQDRDEKIKESLITPENDNVVQYTTEDGEIRTIIWAKGINGPLMGEGGDFHKEIIQGGKDTYITYTVPYSSGDGWYDVNKTTSGGNIDIDKNLCFAAVSSNMLHWWFDQNIEYVDRYIEKNGDIIRANRKLSDLKTSFESQEKSEIFELYKVLYGYNERGFYSDLLMDLFINGYTPKITGATNIESDDLIPSNNGGFFHDVFKGEKLTERTYGGNYQSLSDLLKEIFGNGGIVGVSHKVFRKSNHIVTLWGAEYDLNGKLKAVYVSDSDDQDERSVGMKRYEIRNVGGRAKLSTNETDKSAGAEVGYLHILYLGTNQWNDYFR

SEQ ID NO: 24 - protein, 613 aa, Mediterraneibacter massiliensis
MKNIQKVCMITCMVSVFSFFCGSLGSYAMDAAGTDRVGQVTEYIDEGGEKRTIYWADHITPPKMGGGDSEFQKHEYEQGGTRYVEYIAPYTAGNGWYDVNKTPDQTQDANLCFSAAAANTLHWWLDQNTTYIDRYLAAYPEAPKAEEIRELKGQTPGQHDSKIYARFVEQFANRTTGNWPDILQDQFINGYPPKENGGTNDPEYDGKKLMETGPDKRGGFFYPVFGPDILTQRRFYDFTGNYQSISADMKQFFEQGQIVTLTYKLWESAHVVTVWGAEYDSAGNLSGVYFSDSDDMDEYGMHRYRVVNKKGQAYVTTDMSDDGGGSPITCLTTLSTGTRYWEKVLTPTELELVWGDTQFVYNGSPQIPTLTAGNIADGDDAWLSVKGEGVEVGTYSASAMLSGNDAGKYSLPAEDAGVSFVITQSGTVFEGGVKAYLGTKETTDVQYGDTITIKVSPRATGNAPDSSEPPSVSVKPTNGQVTFFAGGQKLNEAVNTDENGVYTLTYDTKKGALKAGANQLTVKFHDDKNMADHEEKLTIFVKAAEHIPGGEEPPAQEGNGEKAPVYGENGEKADRADRAVKTGDDTSGLIWMFISAGAAAVVYGLYVRNRKKA

SEQ ID NO: 25 - protein, 740 aa, Lachnospiraceae bacterium
MQKFNKILAPAFLGLSMSLLFAVSSYASVEGWKVENGTWKYYKEYKALKSWQKLGNNWYFFNEDGSLKTGWLKDGNDNWYFLDLNSGSNQGVLLSGWQWIDGYCYYFETSDSGTLGRMYADKTVDGYKLNPMGRWVDNNGKELYDATRGISTNKQNLSSDKDLAKKASIAAKRSGSAGGVSRGSGGASSGGGSSRSTGSSYSYSSGNSNFSNSASKHSSDSDNTGSSYSYDDGSLSNSNSNSTKDNLIQSNNNSVSTDNSLNSAGGSSSANVGSSSNSGLSSSLGSVTKPSTGLVSQNQGSLSSDSNNKTNADSKQNTVPDKSNNKKFEDTNTENPKTGNEHSTPPSASENSAGSNTKGSLTPAAEHGDNTDPTEDTTATSSNAAPKPENKEIPNATEDSKKQENENKAKEQEENKADKVKDLLTTEKNNNVVQYTDEDGKIRTIIWAKGISAPIMGEGGDFRKEVTHAGSDTYIDYKAPFTFGNSWYDSNKSRAGGNTDIDKNLCFGATSANMLHWWFEQNSSYIDSYIAKEGDITRSGRSLSELRNSFNNQQDSGIFELFKVLFGYNDKGFYSDLLMDLFINGYTPKISGATNIENEDMTPDNRGGFFYNAFKEVKLTERTYGGSYEDLSEKLKDILGNEGIIGISHKTFGNSSHIVTLWGAEYDLNGKLSAVYVSDSDDQNEEADETDLGMKRYEVRNVGGIAKLSTNQSNKSAGSAIGYLHVLYLGSEQWQSYINQ

SEQ ID NO: 26 - protein, 687 aa, Oribacterium sinus
MGWDQDSQVKDGLAEFRAYHTAEKHSQKLVRNHTQKYIDKTIGARKNGGHPFSVFSRSFMLSIPLALTLPFFSLTAQAEGKWVQAEGQWQYQEEGQNQKGWKEISGSWYYFDPLTGKMQDGWILADGKWYFLKTDTANWGKMAQGWTWVDGYCYFLKDNGTMATEEKTSDGYSISANGQWVQDGKPVHEEGKGVSSRRSAQVEKEIKAGVAEGQQINANGEAQNTGIKGIAGSGGSGGSGGGGGFSGGSGSGGGSSFGGSSSSGGFGSGSGSSFASASGSTSSASGSSASSVGGGFHFGAGNSSGTVESDSRQRDLFGDSKYDSVSNTEDNTGFSPEATEKENTFSEEELARRAEKQRKQAEKELAKRKKLLEKIENGQNNNTVEYETEEGEKRTVLFVKGVKAPKLGENGDFRKTEDHGYIDYKAPYEEGQGYFDVNKAPFGTNKEIDRNLCFAAAASNTLHWYLQQNKKEIEDYIKNNGDVIRTVGANTYSLKDMLNQDVEQQGSLIYQYFKEMYGNNETGYYTVPLMDLFLNGYTPKEDRKTNIENKDLQPDARGGFLYGIIGTKPQTGMHLVNSLSDLGNSLQHYLSNNFVVCLSYTTFSYNHVVTLWGAEYDESGLLRAVYVTDSDDQDETGVETDVAMKRYVVKGNGNLSYLSNAISEEAKGARINSLQYLRFGGEEDLED

SEQ ID NO: 27 - protein, 235 aa, synthetic construct
GQQMETGDQRFGDLVFRQLAPNVWQHTSYLDMPGFGAVASNGLIVRDGGRVLVVDTAWTDDQTAQILNWIKQEINLPVALAVVTHAHQDKMGGMDALHAAGIATYANALSNQLAPQEGMVAAQHSLTFAANGWVEPATAPNFGPLKVFYPGPGHTSDNITVGIDGTDIAFGGCLIKDSKAKSLGNLGDADTEHYAASARAFGAAFPKASMIVMSHSAPDSRAAITHTARMADKLR

SEQ ID NO: 28 - protein, 280 aa, synthetic construct
MKYLLPTAAAGLLLLAAQPAMAMAAHHHHHHSSGVDLGTENLYFQGQQMETGDQRFGDLVFRQLAPNVWQHTSYLDMPGFGAVASNGLIVRDGGRVLVVDTAWTDDQTAQILNWIKQEINLPVALAVVTHAHQDKMGGMDALHAAGIATYANALSNQLAPQEGMVAAQHSLTFAANGWVEPATAPNFGPLKVFYPGPGHTSDNITVGIDGTDIAFGGCLIKDSKAKSLGNLGDADTEHYAASARAFGAAFPKASMIVMSHSAPDSRAAITHTARMADKLR

SEQ ID NO: 29 - protein, 255 aa, synthetic construct
HHHHHHSSGVDLGTENLYFQGQQMETGDQRFGDLVFRQLAPNVWQHTSYLDMPGFGAVASNGLIVRDGGRVLVVDTAWTDDQTAQILNWIKQEINLPVALAVVTHAHQDKMGGMDALHAAGIATYANALSNQLAPQEGMVAAQHSLTFAANGWVEPATAPNFGPLKVFYPGPGHTSDNITVGIDGTDIAFGGCLIKDSKAKSLGNLGDADTEHYAASARAFGAAFPKASMIVMSHSAPDSRAAITHTARMADKLR

SEQ ID NO: 30 - protein, 270 aa, Klebsiella sp.
MELPNIMHPVAKLSTALAAALMLSGCMPGEIRPTIGQQMETGDQRFGDLVFRQLAPNVWQHTSYLDMPGFGAVASNGLIVRDGGRVLVVDTAWTDDQTAQILNWIKQEINLPVALAVVTHAHQDKMGGMDALHAAGIATYANALSNQLAPQEGMVAAQHSLTFAANGWVEPATAPNFGPLKVFYPGPGHTSDNITVGIDGTDIAFGGCLIKDSKAKSLGNLGDADTEHYAASARAFGAAFPKASMIVMSHSAPDSRAAITHTARMADKLR

SEQ ID NO: 31 - protein, 347 aa, synthetic construct
MAEVISGSAVTLNTNMTKNVQNGRAYIDLYDVKNGKIDPLQLITLNSPDLKAQYVIRQGGNYFTQPSELTTVGAASINYTVLKTDGSPHTKPDGQVDIINVSLTIYNSSALRDKIDEVKKKAEDPKWDEGSRDKVLISLDDIKTDIDNNPKTQSDIANKITEVTNLEKILVPRIPEFSTIPGSAATLNTSITKNIQNGNAYIDLYDVKLGKIDPLQLIVLEQGFTAKYVFRQGTKYYGDVSQLQSTGRASLTYNIFGEDGLPHVKTDGQIDIVSVALTIYDSTTLRDKIEEVRTNANDPKWTEESRTEVLTGLDTIKTDIDNNPKTQTDIDSKIVEVNELEKLLVLS

SEQ ID NO: 32 - protein, 347 aa, synthetic construct
MAEVISGSAATLNSALVKNVSGGKAYIDIYDVKNGKIDPLNLIVLTPSNYSANYYIKQGGRIFTSVNQLQTPGTATITYNILDENGNPYTKSDGQIDIVSLVTTVYDTTELRNNINKVIENANDPKWSDDSRKDVLSKIEVIKNDIDNNPKTQSDIDNKIVEVNELEKLLVLPEFSTIPGSAATLNTSITKNIQNGNAYIDLYDVKNGLIDPQNLIVLNPSSYSANYYIKQGAKYYSNPSEITTTGSATITFNILDETGNPHKKADGQIDIVSVNLTIYDSTALRNRIDEVINNANDPKWSDGSRDEVLTGLEKIKKDIDNNPKTQIDIDNKINEVNEIEKLLVVSL